European Patent Specification EP 3 639 854 B1, published January 7, 2026. Title: A medicament for treating or preventing conditions, disorders or diseases of the eye comprising mTOR inhibitors and use of the same. Applicant: The Doshisha. The sequence listing filed with the application follows.

SEQUENCE LISTING (2 sequences)

SEQ ID NO: 1 - DNA, 21 bp, artificial sequence
  Sense strand of siRNA
cauucgcauucaguccauatt

SEQ ID NO: 2 - DNA, 21 bp, artificial sequence
  Antisense strand of siRNA
uauggacugaaugcgaaugat